European Patent Application EP 4 620 530 A2, published September 24, 2025. Title: NEUTRALIZING ANTIBODIES TO GP120 AND THEIR USE. Applicant: The U.S.A. as represented by the Secretary, Department of Health and Human Services National Institutes of Health. Application IB PCT/US2016/023145, filed March 18, 2016. The sequence listing filed with the application follows.

SEQUENCE LISTING (115 sequences)

SEQ ID NO: 1 - protein, 122 aa, Homo sapiens [sequence omitted]

SEQ ID NO: 2 - protein, 103 aa, Homo sapiens [sequence omitted]

SEQ ID NO: 3 - protein, 122 aa, Homo sapiens
RAHLVQSGTAVKRPGASVRVSCETSGYTFTAHILYWFRQAPGRGLEWVGWIKPQYGAVNFGGGFRGRVTLTRDIYRDTAYMDISGLRFDDTAVYYCARDRSYDDSSWALDAWGQGTTVVVSA

SEQ ID NO: 4 - protein, 103 aa, Homo sapiens
YIHVTQSPSSLSVSAGDRVTINCQTSQGVGRDLHWYQHKPGRAPKLLIRHASSVEDGVPSRFSGTGFHTSFNLTINDLQSDDIATYYCQVLESFGRGSRLDFK

SEQ ID NO: 5 - protein, 122 aa, Homo sapiens
QVQLVQSGTAMKKPGASVRVSCQTSGYTFTAHILFWFRQAPGRGLEWVGWIKPQYGAVNFGGGFRDRVTLTRDIYREIAYMDIRGLKLDDTAVYYCARDRSYGDSSWALDAWGQGTTVVASA

SEQ ID NO: 6 - protein, 103 aa, Homo sapiens
YIHVTQSPSSLSVSIGDRVTINCQTSQGVGSDLHWYQHKPGRAPKLLIHHASSVEDGVPSRFSGSGFHTSFNLTINDLQADDIATYYCQVLQFFGRGSRLHIK

SEQ ID NO: 7 - protein, 5 aa, Homo sapiens
AHILF

SEQ ID NO: 8 - protein, 17 aa, Homo sapiens
WIKPQYGAVNFGGGFRD

SEQ ID NO: 9 - protein, 13 aa, Homo sapiens
DRSYGDSSWALDA

SEQ ID NO: 10 - protein, 11 aa, Homo sapiens
QTSQGVGSDLH

SEQ ID NO: 11 - protein, 7 aa, Homo sapiens
HTSSVED

SEQ ID NO: 12 - protein, 5 aa, Homo sapiens
QVLQF

SEQ ID NO: 13 - protein, 5 aa, Homo sapiens
AHILY

SEQ ID NO: 14 - protein, 17 aa, Homo sapiens
WIKPQYGAVNFGGGFRG

SEQ ID NO: 15 - protein, 13 aa, Homo sapiens
DRSYDDSSWALDA

SEQ ID NO: 16 - protein, 11 aa, Homo sapiens
QTSQGVGRDLH

SEQ ID NO: 17 - protein, 7 aa, Homo sapiens
HASSVED

SEQ ID NO: 18 - protein, 5 aa, Homo sapiens
QVLES

SEQ ID NO: 19 - protein, 5 aa, synthetic construct
  REGION 1..5: note = consensus sequence
  SITE 5: note = MISC_FEATURE - X is F or Y
AHILX

SEQ ID NO: 20 - protein, 17 aa, synthetic construct
  REGION 1..17: note = consensus sequence
  SITE 17: note = MISC_FEATURE - X is D or G
WIKPQYGAVNFGGGFRX

SEQ ID NO: 21 - protein, 16 aa, synthetic construct
  REGION 1..16: note = consensus sequence
  SITE 7: note = MISC_FEATURE - X is G or D
ARDRSYXDSSWALDAW

SEQ ID NO: 22 - protein, 11 aa, synthetic construct
  REGION 1..11: note = consensus sequence
  SITE 8: note = MISC_FEATURE - X is G or S
QTSQGVGXDLH

SEQ ID NO: 23 - protein, 7 aa, synthetic construct
  REGION 1..7: note = consensus sequence
  SITE 2: note = MISC_FEATURE - X is A or T
HXSSVED

SEQ ID NO: 24 - protein, 6 aa, synthetic construct
  REGION 1..6: note = consensus sequence
  SITE 4: note = MISC_FEATURE - X is E or Q
  SITE 5: note = MISC_FEATURE - X is S or F
QVLXXF

SEQ ID NO: 25 - protein, 15 aa, synthetic construct
  REGION 1..15: note = CAR sequence
GGGGSGGGGSGGGGS

SEQ ID NO: 26 - protein, 22 aa, synthetic construct
  REGION 1..22: note = CAR sequence
LLVTSLLLCELPHPAFLLIPDT

SEQ ID NO: 27 - protein, 236 aa, synthetic construct
  REGION 1..236: note = CAR sequence
EPKSCDKTHTCPPCPAPELLGGPSVFLFPPKPKDTLMISRTPEVTCVVVDVSHEDPEVKFNWYVDGVEVHNAKTKPREEQYNSTYRVVSVLTVLHQDWLNGKEYKCKVSNKALPAPIEKTISKAKGQPREPQVYTLPPSRDELTKNQVSLTCLVKGFYPSDIAVEWESNGQPENNYKTTPPVLDSDGSFFLYSKLTVDKSRWQQGNVFSCSVMHEALHNHYTQKSLSLSPGKKDPK

SEQ ID NO: 28 - protein, 69 aa, synthetic construct
  REGION 1..69: note = CAR sequence
TTTPAPRPPTPAPTIASQPLSLRPEACRPAAGGAVHTRGLDFACDIYIWAPLAGTCGVLLLSLVITLYC

SEQ ID NO: 29 - protein, 67 aa, synthetic construct
  REGION 1..67: note = CAR sequence
IEVMYPPPYLDNEKSNGTIIHVKGKHLCPSPLFPGPSKPFWVLVVVGGVLACYSLLVTVAFIIFWVR

SEQ ID NO: 30 - protein, 112 aa, synthetic construct
  REGION 1..112: note = CAR sequence
RVKFSRSADAPAYQQGQNQLYNELNLGRREEYDVLDKRRGRDPEMGGKPRRKNPQEGLYNELQKDKMAEAYSEIGMKGERRRGKGHDGLYQGLSTATKDTYDALHMQALPPR

SEQ ID NO: 31 - protein, 84 aa, synthetic construct
  REGION 1..84: note = CAR sequence
FVPVFLPAKPTTTPAPRPPTPAPTIASQPLSLRPEACRPAAGGAVHTRGLDFACDIYIWAPLAGTCGVLLLSLVITLYCNHRNR

SEQ ID NO: 32 - protein, 40 aa, synthetic construct
  REGION 1..40: note = CAR sequence
SKRSRLLHSDYMNMTPRRPGPTRKHYQPYAPPRDFAAYRS

SEQ ID NO: 33 - protein, 42 aa, synthetic construct
  REGION 1..42: note = CAR sequence
KRGRKKLLYIFKQPFMRPVQTTQEEDGCSCRFPEEEEGGCEL

SEQ ID NO: 34 - protein, 47 aa, synthetic construct
  REGION 1..47: note = CAR sequence
RFSVVKRGRKKLLYIFKQPFMRPVQTTQEEDGCSCRFPEEEEGGCEL

SEQ ID NO: 35 - protein, 856 aa, Human immunodeficiency virus 1
MRVKEKYQHLWRWGWRWGTMLLGMLMICSATEKLWVTVYYGVPVWKEATTTLFCASDAKAYDTEVHNVWATHACVPTDPNPQEVVLVNVTENFNMWKNDMVEQMHEDIISLWDQSLKPCVKLTPLCVSLKCTDLKNDTNTNSSSGRMIMEKGEIKNCSFNISTSIRGKVQKEYAFFYKLDIIPIDNDTTSYKLTSCNTSVITQACPKVSFEPIPIHYCAPAGFAILKCNNKTFNGTGPCTNVSTVQCTHGIRPVVSTQLLLNGSLAEEEVVIRSVNFTDNAKTIIVQLNTSVEINCTRPNNNTRKRIRIQRGPGRAFVTIGKIGNMRQAHCNISRAKWNNTLKQIASKLREQFGNNKTIIFKQSSGGDPEIVTHSFNCGGEFFYCNSTQLFNSTWFNSTWSTEGSNNTEGSDTITLPCRIKQIINMWQKVGKAMYAPPISGQIRCSSNITGLLLTRDGGNSNNESEIFRPGGGDMRDNWRSELYKYKVVKIEPLGVAPTKAKRRVVQREKRAVGIGALFLGFLGAAGSTMGAASMTLTVQARQLLSGIVQQQNNLLRAIEAQQHLLQLTVWGIKQLQARILAVERYLKDQQLLGIWGCSGKLICTTAVPWNASWSNKSLEQIWNHTTWMEWDREINNYTSLIHSLIEESQNQQEKNEQELLELDKWASLWNWFNITNWLWYIKLFIMIVGGLVGLRIVFAVLSIVNRVRQGYSPLSFQTHLPTPRGPDRPEGIEEEGGERDRDRSIRLVNGSLALIWDDLRSLCLFSYHRLRDLLLIVTRIVELLGRRGWEALKYWWNLLQYWSQELKNSAVSLLNATAIAVAEGTDRVIEVVQGACRAIRHIPRRIRQGLERILL

SEQ ID NO: 36 - DNA, 366 bp, Homo sapiens
  source 1..366: mol_type = other DNA
cgagcgcacctggtacaatcagggactgcgatgaagaaaccgggggcctcagtaagagtctcctgccagacctctggatacacctttaccgcccacatattattttggttccgacaggcccccgggcgaggacttgagtgggtggggtggatcaagccacaatatggggccgtgaattttggtggtggttttcgggacagggtcacattgactcgagacgtatatagagagattgcgtacatggacatcagaggccttaaacctgacgacacggccgtctattactgtgcgagagaccgttcctatggcgactcctcttgggccttagatgcctggggacagggaacgacggtcgtcgtctccgcg

SEQ ID NO: 37 - DNA, 309 bp, Homo sapiens
  source 1..309: mol_type = other DNA
tacatccacgtgacccagtctccgtcctccctgtctgtgtctattggagacagagtcaccatcaattgccagacgagtcagggtgttggcagtgacctacattggtatcaacacaaaccggggagagcccctaaactcttgatccaccatacctcttctgtggaagacggtgtcccctcaagattcagcggctctggatttcacacatcttttaatctgaccatcagcgacctacaggctgacgacattgccacatattactgtcaagttttacaatttttcggccgagggagtcgactccatattaaa

SEQ ID NO: 38 - DNA, 366 bp, Homo sapiens
  source 1..366: mol_type = other DNA
cgagcgcacctggtacaatcagggactgcggtgaagagaccgggggcctcagtaagggtctcctgcgagacttctggatacacctttaccgcccacatattatactggttccgacaggcccccgggcgagggcttgagtgggtggggtggatcaagccacaatacggtgccgtgaactttgggggtggttttcggggcagggtcacattgacgcgagacatatatagagatactgcatatatggacatcagtggcctgagatttgacgacacggccgtctactattgtgcgagagaccgttcttatgacgactcttcttgggccttagatgcctggggccagggaacgacggtcgtcgtctccgcg

SEQ ID NO: 39 - DNA, 309 bp, Homo sapiens
  source 1..309: mol_type = other DNA
tacatccacgtgacccagtctccgtcctccctgtctgtgtctgctggggacagagtcaccatcaattgccagacgagtcagggtgttggccgtgacctacattggtatcaacacaaaccggggagagcccctaaactcctgatccgccacgcctcttctgtggaggacggtgtcccgtcaagattcagtggcactggatttcacacatcttttaatttgaccatcaacgacctgcagtctgacgacattgccacatattactgtcaggtgttagaatctttcggccgagggagtcgactggattttaaa

SEQ ID NO: 40 - DNA, 366 bp, Homo sapiens
  source 1..366: mol_type = other DNA
caggtgcagctggtacaatcagggactgcgatgaagaaaccgggggcctcagtaagggtctcctgccagacttctggatacacctttaccgcccacatattattttggttccgacaggcccccgggcgagggcttgagtgggtgggatggatcaagccacaatacggggccgtgaattttggtggtggttttcgggacagggtcacattgactcgagacatatatagagagattgcatacatggacatcagaggccttaaacttgacgacacggccgtctattactgtgcgagagaccgttcctatggcgactcctcttgggccttagatgcctggggacagggaacgacggtcgtcgcctccgcg

SEQ ID NO: 41 - DNA, 309 bp, Homo sapiens
  source 1..309: mol_type = other DNA
tacatccacgtgacccagtctccgtcctccctgtctgtgtctattggagacagagtcaccatcaattgccagacgagtcagggtgttggcagtgacctacattggtatcaacacaaaccggggagagcccctaaactcttgatccaccatgcctcttctgtggaggacggtgtcccgtcaagattcagtggctctggatttcacacatcttttaatctgaccatcaacgacctacaggctgacgacattgccacatattactgtcaggttttacaatttttcggccgagggagtcgactccatattaaa

SEQ ID NO: 42 - protein, 121 aa, synthetic construct
  REGION 1..121: note = variant antibody sequence
QVQLVQSGGQMKKPGESMRISCRASGYEFIDCTLNWIRLAPGKRPEWMGWLKPRYGAVNYARPLQGRVTMTRDVYSDTAFLELRSLTVDDTAVYFCTRGKNCDYNWDFEHWGRGTPVIVSS

SEQ ID NO: 43 - protein, 121 aa, synthetic construct
  REGION 1..121: note = variant antibody sequence
QVQLVQSGGQMKKPGESMRISCRASGYEFIDCTLNWIRLAPGKRPEWMGWLKPRGGAVNYGGGLQGRVTMTRDVYSDTAFLELRSLTVDDTAVYFCTRGKNCDYNWDFEHWGRGTPVIVSS

SEQ ID NO: 44 - protein, 122 aa, synthetic construct
  REGION 1..122: note = variant antibody sequence
QVQLVQSGGQMKKPGESMRISCRASGYEFIDCTLNWIRLAPGKRPEWMGWLKPRGGAVNYARPLQGRVTMTRDVYSDTAFLELRSLTVDDTAVYFCARDRSYGDSSWALDAWGRGTPVIVSS

SEQ ID NO: 45 - protein, 122 aa, synthetic construct
  REGION 1..122: note = variant antibody sequence
QVRLSQSGGQMKKPGDSMRISCRASGYEFINCPINWIRLAPGKRPEWMGWMKPRHGAVSYARQLQGRVTMTRDMYSETAFLELRSLTSDDTAVYFCARDRSYGDSSWALDAWGQGTPVTVSS

SEQ ID NO: 46 - protein, 122 aa, synthetic construct
  REGION 1..122: note = variant antibody sequence
QVQLVQSGTQMKEPGASVTISCVTSGYEFVEILINWVRQVPGRGLEWMGWMNPRGGGVNYARQFQGKVTMTRDVYRDTAYLTLSGLTSGDTAKYFCARDRSYGDSSWALDAWGQGTLVIVSP

SEQ ID NO: 47 - protein, 122 aa, synthetic construct
  REGION 1..122: note = variant antibody sequence
RAHLVQSGTAMKKPGASVRVSCQTSGYTFTAHILFWFRQAPGRGLEWVGWIKPQGGAVNFGGGFRDRVTLTRDVYREIAYMDIRGLKPDDTAVYYCARDRSYGDSSWALDAWGQGTTVVVSA

SEQ ID NO: 48 - protein, 122 aa, synthetic construct
  REGION 1..122: note = variant antibody sequence
RAHLVQSGTAMKKPGASVRVSCQTSGYTFTAHILFWFRQAPGRGLEWVGWIKPQYGAVNFARPFRDRVTLTRDVYREIAYMDIRGLKPDDTAVYYCARDRSYGDSSWALDAWGQGTTVVVSA

SEQ ID NO: 49 - protein, 125 aa, synthetic construct
  REGION 1..125: note = variant antibody sequence
RAHLVQSGTAMKKPGASVRVSCQTSGYTFTAHILFWFRQAPGRGLEWVGWIKPQYGAVNFGGGFRDRVTLTRDVYREIAYMDIRGLKPDDTAVYYCARGKYCTARDYYNWALDAWGQGTTVVVSA

SEQ ID NO: 50 - protein, 132 aa, synthetic construct
  REGION 1..132: note = variant antibody sequence
RAHLVQSGTAMKKPGASVRVSCQTSGYTFTAHILFWFRQAPGRGLEWVGWIKPQYGAVNFGGGFRDRVTLTRDVYREIAYMDIRGLKPDDTAVYYCARGRSCCGGRRHCNGADCFNWALDAWGQGTTVVVSA

SEQ ID NO: 51 - protein, 122 aa, synthetic construct
  REGION 1..122: note = variant antibody sequence
RAHLVQSGTAMKKPGASVRVSCQTSGYTFTAHILFWFRQAPGRGLEWVGWIKPKFGAVNYAHSFQGRVTLTRDVYREIAYMDIRGLKPDDTAVYYCARDRSYGDSSWALDAWGQGTTVVVSA

SEQ ID NO: 52 - protein, 122 aa, synthetic construct
  REGION 1..122: note = variant antibody sequence
RAHLVQSGTAMKKPGASVRVSCQTSGYTFTAHILFWFRQAPGRGLEWVGWIKPQYGAVNFGGGFRDRVTLTRDVYREIAYMDIRGLKPDDTAVYYCARDRLYDGSSWRLDPWGQGTTVVVSA

SEQ ID NO: 53 - protein, 122 aa, synthetic construct
  REGION 1..122: note = variant antibody sequence
SQRLVQSGPQVRKPGSSVRISCETSGYTFNAHILFWFRQAPGRGLEWVGWIKPQYGAVNFGGGFRDRVTLTRDVYREIAYMDIRGLKPDDTAVYYCARDRSYGDSSWALDAWGQGTTVVVSA

SEQ ID NO: 54 - protein, 122 aa, synthetic construct
  REGION 1..122: note = variant antibody sequence
RAHLVQSGTAMKKPGASVRVSCQTSGYTFTAHILFWFRQAPGRSFEWMGWIKPQYGAVNFGGGFRDRVTLTRDVYREIAYMDIRGLKPDDTAVYYCARDRSYGDSSWALDAWGQGTTVVVSA

SEQ ID NO: 55 - protein, 122 aa, synthetic construct
  REGION 1..122: note = variant antibody sequence
RAHLVQSGTAMKKPGASVRVSCQTSGYTFTAHILFWFRQAPGRGLEWVGWIKPQYGAVNFGGGFRDRITLTRDIYRETAFLDLTGLRFDDTAVYYCARDRSYGDSSWALDAWGQGTTVVVSA

SEQ ID NO: 56 - protein, 122 aa, synthetic construct
  REGION 1..122: note = variant antibody sequence
RAHLVQSGTAVKRPGASVRVSCETSGYTFTAHILFWFRQAPGRGLEWVGWIKPQYGAVNFGGGFRDRVTLTRDVYREIAYMDIRGLKPDDTAVYYCARDRSYGDSSWALDAWGQGTTVVVSA

SEQ ID NO: 57 - protein, 122 aa, synthetic construct
  REGION 1..122: note = variant antibody sequence
RAHLVQSGTAMKKPGASVRVSCQTSGYTFTAHILFWFRQAPGRGLEWVGWIKPQYGAVNFGGGFRDRVTLTRDIYRDTAYMDISGLRFDDTAVYYCARDRSYGDSSWALDAWGQGTTVVVSA

SEQ ID NO: 58 - protein, 103 aa, synthetic construct
  REGION 1..103: note = variant antibody sequence
YIHVTQSPSSLSVSAGDRVTINCQTSQGVGSDLHWYQHKPGRAPKLLIHHTSSVEDGVPSRFSGSGFHTSFNLTISDLQADDIATYYCQVLQFFGRGSRLHIK

SEQ ID NO: 59 - protein, 103 aa, synthetic construct
  REGION 1..103: note = variant antibody sequence
YIHVTQSPSSLSVSIGDRVTINCQTSQGVGSDLHWYQHKPGRAPKLLIRHTSSVEDGVPSRFSGSGFHTSFNLTISDLQADDIATYYCQVLQFFGRGSRLHIK

SEQ ID NO: 60 - protein, 103 aa, synthetic construct
  REGION 1..103: note = variant antibody sequence
YIHVTQSPSSLSVSIGDRVTINCQTSQGVGSDLHWYQHKPGRAPKLLIHHTSSVEDGVPSRFSGTGFHTSFNLTINDLQSDDIATYYCQVLQFFGRGSRLHIK

SEQ ID NO: 61 - protein, 103 aa, synthetic construct
  REGION 1..103: note = variant antibody sequence
YIHVTQSPSSLSVSIGDRVTINCQTSQGVGSDLHWYQHKPGRAPKLLIHHTSSVEDGVPSRFSGSGFHTSFNLTISDLQADDIATYYCQVLQFFGRGSRLDFK

SEQ ID NO: 62 - protein, 103 aa, synthetic construct
  REGION 1..103: note = variant antibody sequence
YIHVTQSPSSLSVSIGDRVTINCQTSQGVGRDLHWYQHKPGRAPKLLIHHTSSVEDGVPSRFSGSGFHTSFNLTISDLQADDIATYYCQVLQFFGRGSRLHIK

SEQ ID NO: 63 - protein, 103 aa, synthetic construct
  REGION 1..103: note = variant antibody sequence
YIHVTQSPSSLSVSIGDRVTINCQTSQGVGSDLHWYQHKPGRAPKLLIHHASSVEDGVPSRFSGSGFHTSFNLTISDLQADDIATYYCQVLQFFGRGSRLHIK

SEQ ID NO: 64 - protein, 103 aa, synthetic construct
  REGION 1..103: note = variant antibody sequence
YIHVTQSPSSLSVSIGDRVTINCQTSQGVGSDLHWYQHKPGRAPKLLIHHTSSVEDGVPSRFSGSGFHTSFNLTISDLQADDIATYYCQVLESFGRGSRLHIK

SEQ ID NO: 65 - DNA, 24 bp, synthetic construct
  misc_feature 1..24: note = oligonucleotide primer
  source 1..24: mol_type = other DNA
ttgctacttgtgattgctccatgt

SEQ ID NO: 66 - DNA, 25 bp, synthetic construct
  misc_feature 1..25: note = oligonucleotide primer
  source 1..25: mol_type = other DNA
tagagccctggaagcatccaggaag

SEQ ID NO: 67 - DNA, 24 bp, synthetic construct
  misc_feature 1..24: note = oligonucleotide primer
  source 1..24: mol_type = other DNA
ttgctacttgtgattgctccatgt

SEQ ID NO: 68 - DNA, 31 bp, synthetic construct
  misc_feature 1..31: note = oligonucleotide primer
  source 1..31: mol_type = other DNA
caccttaggcatctcctatggcaggaagaag

SEQ ID NO: 69 - DNA, 23 bp, synthetic construct
  misc_feature 1..23: note = oligonucleotide primer
  source 1..23: mol_type = other DNA
gtctcgagatactgctcccaccc

SEQ ID NO: 70 - DNA, 18 bp, synthetic construct
  misc_feature 1..18: note = oligonucleotide primer
  source 1..18: mol_type = other DNA
caccatggcaggaagaag

SEQ ID NO: 71 - DNA, 23 bp, synthetic construct
  misc_feature 1..23: note = oligonucleotide primer
  source 1..23: mol_type = other DNA
gtctcgagatactgctcccaccc

SEQ ID NO: 72 - protein, 8 aa, synthetic construct
  REGION 1..8: note = synthetic peptide
AFILMYWV

SEQ ID NO: 73 - protein, 121 aa, Homo sapiens
QVQLVQSGGQMKKPGESMRISCRASGYEFIDCTLNWIRLAPGKRPEWMGWLKPRGGAVNYARPLQGRVTMTRDVYSDTAFLELRSLTVDDTAVYFCTRGKNCDYNWDFEHWGRGTPVIVSS

SEQ ID NO: 74 - protein, 104 aa, Homo sapiens
EIVLTQSPGTLSLSPGETAIISCRTSQYGSLAWYQQRPGQAPRLVIYSGSTRAAGIPDRFSGSRWGPDYNLTISNLESGDFGVYYCQQYEFFGQGTKVQVDIKR

SEQ ID NO: 75 - protein, 121 aa, Homo sapiens
QRLVQSGPQVRKPGSSVRISCETSGYTFNAYILHWFRQAPGRSFEWMGWIKPKFGAVNYAHSFQGRITLTRDIYRETAFLDLTGLRFDDTAVYYCARDRLYDGSSWRLDPWGQGTRVVVSS

SEQ ID NO: 76 - protein, 103 aa, Homo sapiens
FALMTQSPATLAVSVGDRVTITCRASQGIGSDLHWYQQKPGRPPKILIHHASAREEGVPSRFGGSGSHTSFIFTINDLQLDDVATYYCQVLESFGQGTRLDIN

SEQ ID NO: 77 - protein, 122 aa, Homo sapiens
QVQLVQSGAEVKKPGASVKVSCKASGYTFTGYYMHWVRQAPGQGLEWMGWINPNSGGTNYAQKFQGRVTMTRDTSISTAYMELSRLRSDDTAVYYCARAYCGGDCYNWFDSWGQGTLVTVSS

SEQ ID NO: 78 - protein, 107 aa, Homo sapiens
DIQMTQSPSSLSASVGDRVTITCQASQDISNYLNWYQQKPGKAPKLLIYDASNLETGVPSRFSGSGSGTDFTFTISSLQPEDIATYYCQQYDNLPITFGQGTRLEIK

SEQ ID NO: 79 - protein, 122 aa, Homo sapiens
RGHLVQSGTEVKKPGASVRVSCETSGYTFTAYILHWFRQAPGRGLEWMGWIKPKYGAVNYAHAFQGRVTLTRDIYRDTAYMDLSGLRFDDTAVYYCARDRVYDDSSWQLDPWGQGTSVIVSS

SEQ ID NO: 80 - protein, 121 aa, Homo sapiens
RGHLVQSGTEVKKPGASVRVSCETSGYTFTAHILHWFRQAPGRGLEWMGWIKPKYGAVNYAHAFQGRVTLTRDIYRDTAYMDLSGLRFDDTAVYYCARDRVYDDSSWQLDPWGQGTSVIVS

SEQ ID NO: 81 - protein, 122 aa, Homo sapiens
RAHLVQSGTAVKKPGASVRVSCQTSGYTFTAHILYWFRQAPGRGLEWVGWIKPQYGAVNFGGGFRGRVTLTRDIYRDTAYMDISGLRFDDTAVYYCARDRSYDDSSWALDAWGQGTTVVVSA

SEQ ID NO: 82 - protein, 122 aa, Homo sapiens
RAHLVQSGTAMKKPGASVRVSCQTSGYTFTAHILFWFRQAPGRGLEWVGWIKPQYGAVNFGGGFRGRVTLTRDVYREIAYMDIRGLKLDDTAVYYCARDRSYGDSSWALDAWGQGTTVVVSA

SEQ ID NO: 83 - protein, 122 aa, Homo sapiens
SQRLVQSGPQVKKPGSSVRISCETSGYTFTAYILHWFRQAPGRSLEWMGWIKPKFGAVNYAHSFQGRITLTRDIYREIAFLDLTGLRFDDTAVYYCARDRLYDGSSWRLDPWGQGTRVIVSS

SEQ ID NO: 84 - protein, 102 aa, Homo sapiens
YIQVTQSPSSLSVSVGDRVTITCQASQGVGNDLHWYQQKPGRAPKLLIYDASTLEAGVPSRFSGSGFHTSFTFTINGLQPDDIATYYCQVLESFGQGTRLEI

SEQ ID NO: 85 - protein, 102 aa, Homo sapiens
YIHVTQSPSSLSVSVGDRVTITCQASQGVGNDLHWYQQKPGRAPKLLIYDASTLEEGVPSRFSGTGFHTSFTFTINGLQPDDIATYYCQVLESFGQGTRLEI

SEQ ID NO: 86 - protein, 102 aa, Homo sapiens
YIHVTQSPSSLSVSVGDRVTITCQASQGVGSDLHWYQQKPGRAPKLLIHHASTLEEGVPSRFSGTGFHTSFTFTINDLQPDDIATYYCQVLESFGQGTRLEI

SEQ ID NO: 87 - protein, 102 aa, Homo sapiens
YIHVTQSPSSLSVSVGDRVTINCQTSQGVGSDLHWYQHKPGRAPKLLIHHASSVEDGVPSRFSGTGFHTSFNLTINDLQADDIATYYCQVLESFGRGSRLDI

SEQ ID NO: 88 - protein, 102 aa, Homo sapiens
YIHVTQSPSSLSVSIGDRVTINCQTSQGVGSDLHWYQHKPGRAPKLLIHHASSVEDGVPSRFSGTGFHTSFNLTINDLQADDIATYYCQVLQSFGRGSRLDI

SEQ ID NO: 89 - protein, 102 aa, Homo sapiens
YIHVTQSPSSLSVSIGDRVTINCQTSQGVGSDLHWYQHKPGRAPKLLIHHASSVEDGVPSRFSGSGFHTSFNLTINDLQADDIATYYCQVLQFFGRGSRLHI

SEQ ID NO: 90 - protein, 102 aa, Homo sapiens
YIHVTQSPSSLAVSVGDRVTITCQASQGVGSDLHWYQHKRGRPPKILIHHASAREEGVPSRFSGSGFHTSFTFTINDLQPDDIATYYCQVLESFGQGTRLEI

SEQ ID NO: 91 - protein, 102 aa, Homo sapiens
YIHVTQSPSSLAVSVGDRVTITCQASQGVGSDLHWYQHKRGRPPKILIHHASAREEGVPSRFSGSGFHTSFTFTINDLQPDDFATYYCQVLESFGQGTRLEI

SEQ ID NO: 92 - protein, 102 aa, Homo sapiens
YIHVTQSPSSLAVSVGDRVTITCRASQGVGSDLHWYQHKRGRPPKILIHHASAREEGVPSRFSGSGFHTSFTFTINDLQPDDFATYYCQVLESFGQGTRLEI

SEQ ID NO: 93 - protein, 102 aa, Homo sapiens
YIHVTQSPSSLAVSVGDRVTITCRASQGIGSDLHWYQHKRGRPPKILIHHASAREEGVPSRFSGSGFHTSFTFTINDLQPDDVATYYCQVLESFGQGTRLDI

SEQ ID NO: 94 - protein, 452 aa, synthetic construct
  REGION 1..452: note = antibody heavy chain
RAHLVQSGTAMKKPGASVRVSCQTSGYTFTAHILFWFRQAPGRGLEWVGWIKPQYGAVNFGGGFRDRVTLTRDVYREIAYMDIRGLKPDDTAVYYCARDRSYGDSSWALDAWGQGTTVVVSAASTKGPSVFPLAPSSKSTSGGTAALGCLVKDYFPEPVTVSWNSGALTSGVHTFPAVLQSSGLYSLSSVVTVPSSSLGTQTYICNVNHKPSNTKVDKKVEPKSCDKTHTCPPCPAPELLGGPSVFLFPPKPKDTLMISRTPEVTCVVVDVSHEDPEVKFNWYVDGVEVHNAKTKPREEQYNSTYRVVSVLTVLHQDWLNGKEYKCKVSNKALPAPIEKTISKAKGQPREPQVYTLPPSRDELTKNQVSLTCLVKGFYPSDIAVEWESNGQPENNYKTTPPVLDSDGSFFLYSKLTVDKSRWQQGNVFSCSVMHEALHNHYTQKSLSLSPGK

SEQ ID NO: 95 - DNA, 1356 bp, synthetic construct
  misc_feature 1..1356: note = antibody heavy chain
  source 1..1356: mol_type = other DNA
cgagcgcacctggtacaatcagggactgcgatgaagaaaccgggggcctcagtaagagtctcctgccagacctctggatacacctttaccgcccacatattattttggttccgacaggcccccgggcgaggacttgagtgggtggggtggatcaagccacaatatggggccgtgaattttggtggtggttttcgggacagggtcacattgactcgagacgtatatagagagattgcgtacatggacatcagaggccttaaacctgacgacacggccgtctattactgtgcgagagaccgttcctatggcgactcctcttgggccttagatgcctggggacagggaacgacggtcgtcgtctccgcggcgtcgaccaagggcccatcggtcttccccctggcaccctcctccaagagcacctctgggggcacagcggccctgggctgcctggtcaaggactacttccccgaaccggtgacggtgtcgtggaactcaggcgccctgaccagcggcgtgcacaccttcccggctgtcctacagtcctcaggactctactccctcagcagcgtggtgaccgtgccctccagcagcttgggcacccagacctacatctgcaacgtgaatcacaagcccagcaacaccaaggtggacaagaaagttgagcccaaatcttgtgacaaaactcacacatgcccaccgtgcccagcacctgaactcctggggggaccgtcagtcttcctcttccccccaaaacccaaggacaccctcatgatctcccggacccctgaggtcacatgcgtggtggtggacgtgagccacgaagaccctgaggtcaagttcaactggtacgtggacggcgtggaggtgcataatgccaagacaaagccgcgggaggagcagtacaacagcacgtaccgtgtggtcagcgtcctcaccgtcctgcaccaggactggctgaatggcaaggagtacaagtgcaaggtctccaacaaagccctcccagcccccatcgagaaaaccatctccaaagccaaagggcagccccgagaaccacaggtgtacaccctgcccccatcccgggatgagctgaccaagaaccaggtcagcctgacctgcctggtcaaaggcttctatcccagcgacatcgccgtggagtgggagagcaatgggcagccggagaacaactacaagaccacgcctcccgtgctggactccgacggctccttcttcctctacagcaagctcaccgtggacaagagcaggtggcagcaggggaacgtcttctcatgctccgtgatgcatgaggctctgcacaaccactacacgcagaagagcctctccctgtctccgggtaaa

SEQ ID NO: 96 - protein, 210 aa, Homo sapiens
YIHVTQSPSSLSVSIGDRVTINCQTSQGVGSDLHWYQHKPGRAPKLLIHHTSSVEDGVPSRFSGSGFHTSFNLTISDLQADDIATYYCQVLQFFGRGSRLHIKRTVAAPSVFIFPPSDEQLKSGTASVVCLLNNFYPREAKVQWKVDNALQSGNSQESVTEQDSKDSTYSLSSTLTLSKADYEKHKVYACEVTHQGLSSPVTKSFNRGEC

SEQ ID NO: 97 - DNA, 630 bp, Homo sapiens
  source 1..630: mol_type = other DNA
tacatccacgtgacccagtctccgtcctccctgtctgtgtctattggagacagagtcaccatcaattgccagacgagtcagggtgttggcagtgacctacattggtatcaacacaaaccggggagagcccctaaactcttgatccaccatacctcttctgtggaagacggtgtcccctcaagattcagcggctctggatttcacacatcttttaatctgaccatcagcgacctacaggctgacgacattgccacatattactgtcaagttttacaatttttcggccgagggagtcgactccatattaaacgtacggtggctgcaccatctgtcttcatcttcccgccatctgatgagcagttgaaatctggaactgcctctgttgtgtgcctgctgaataacttctaccccagagaagccaaagtgcagtggaaggtggacaacgccctgcagagcggaaacagccaggaaagcgtgacagagcaggattccaaggattccacatacagcctgagcagcacactgacactgtccaaggccgactacgagaagcacaaggtgtacgcctgcgaagtgacacaccagggactgtcctcccctgtgacaaagagcttcaacagaggagaatgc

SEQ ID NO: 98 - protein, 452 aa, Homo sapiens
RAHLVQSGTAMKKPGASVRVSCQTSGYTFTAHILFWFRQAPGRGLEWVGWIKPQYGAVNFGGGFRDRVTLTRDVYREIAYMDIRGLKPDDTAVYYCARDRSYGDSSWALDAWGQGTTVVVSAASTKGPSVFPLAPSSKSTSGGTAALGCLVKDYFPEPVTVSWNSGALTSGVHTFPAVLQSSGLYSLSSVVTVPSSSLGTQTYICNVNHKPSNTKVDKRVEPKSCDKTHTCPPCPAPELLGGPSVFLFPPKPKDTLMISRTPEVTCVVVDVSHEDPEVKFNWYVDGVEVHNAKTKPREEQYNSTYRVVSVLTVLHQDWLNGEEYKCKVSNKALPAPIEKTISKAKGQPREPQVYTLPPSREEMTKNQVSLTCLVKGFYPSDIAVEWESNGQPENNYKTTPPVLDSDGSFFLYSKLTVDKSRWQQGNVFSCSVMHEALHNHYTQKSLSLSPGK

SEQ ID NO: 99 - DNA, 1356 bp, Homo sapiens
  source 1..1356: mol_type = other DNA
cgagcgcacctggtacaatcagggactgcgatgaagaaaccgggggcctcagtaagagtctcctgccagacctctggatacacctttaccgcccacatattattttggttccgacaggcccccgggcgaggacttgagtgggtggggtggatcaagccacaatatggggccgtgaattttggtggtggttttcgggacagggtcacattgactcgagacgtatatagagagattgcgtacatggacatcagaggccttaaacctgacgacacggccgtctattactgtgcgagagaccgttcctatggcgactcctcttgggccttagatgcctggggacagggaacgacggtcgtcgtctccgcggcctccaccaagggcccatcggtcttccccctggcaccctcctccaagagcacctctgggggcacagcggccctgggctgcctggtcaaggactacttccccgaaccggtgacggtgtcgtggaactcaggcgccctgaccagcggcgtgcacaccttcccggctgtcctacagtcctcaggactctactccctcagcagcgtggtgaccgtgccctccagcagcttgggcacccagacctacatctgcaacgtgaatcacaagcccagcaacaccaaggtggacaagagagttgagcccaaatcttgtgacaaaactcacacatgcccaccgtgcccagcacctgaactcctggggggaccgtcagtcttcctcttccccccaaaacccaaggacaccctcatgatctcccggacccctgaggtcacatgcgtggtggtggacgtgagccacgaagaccctgaggtcaagttcaactggtacgtggacggcgtggaggtgcataatgccaagacaaagccgcgggaggagcagtacaacagcacgtaccgtgtggtcagcgtcctcaccgtcctgcaccaggactggctgaatggcgaggagtacaagtgcaaggtctccaacaaagccctcccagcccccatcgagaaaaccatctccaaagccaaagggcagccccgagaaccacaggtgtacaccctgcccccatcccgggaggagatgaccaagaaccaggtcagcctgacctgccttgtcaaaggcttctatcccagcgacatcgccgtggagtgggagagcaatgggcagccggagaacaactacaagaccacgcctcccgtgctggactccgacggctccttcttcctctacagcaagctcaccgtggacaagagcaggtggcagcaggggaacgtcttctcatgctccgtgatgcatgaggctctgcacaaccactacacgcagaagagcctctccctgtctccgggtaaa

SEQ ID NO: 100 - DNA, 366 bp, Homo sapiens
  source 1..366: mol_type = other DNA
cgagggcacttggtgcagtcagggactgaggtgaagaaaccgggggcctcagtgagagtctcctgcgagacttctggatacaccttcaccgcctacattttacattggttccgacaggcccccggacgagggcttgagtggatggggtggatcaagccaaaatatggagccgtcaattatgctcatgcatttcagggcagggtcaccctgaccagagacatatatagagacactgcatacatggacttgagtggcctaagattcgacgacacggccgtctattactgtgcgagagatcgcgtttatgacgattcgtcttggcaattggatccctggggccagggaacttcggtcatcgtctcctca

SEQ ID NO: 101 - DNA, 366 bp, Homo sapiens
  source 1..366: mol_type = other DNA
cgagggcacttggtgcagtcagggactgaggtgaagaaaccgggggcctcagtgagagtctcctgcgagacttctggatacaccttcaccgcccacattttacattggttccgacaggcccccggacgagggcttgagtggatggggtggatcaagccaaaatatggagccgtcaattatgctcatgcatttcagggcagggtcaccctgaccagagacatatatagagacactgcatacatggacttgagtggcctaagattcgacgacacggccgtctattactgtgcgagagatcgcgtttatgacgattcgtcttggcaattggatccctggggccagggaacttcggtcatcgtctcctca

SEQ ID NO: 102 - DNA, 366 bp, Homo sapiens
  source 1..366: mol_type = other DNA
cgagcgcacttggtgcagtcagggactgcggtgaagaaaccgggggcctcagtgagagtctcctgcgagacttctggatacaccttcaccgcccacattttatattggttccgacaggcccccggacgagggcttgagtgggtggggtggatcaagccacaatatggggccgtgaattttggtggtggttttcggggcagggtcaccctgaccagagacatatatagagacactgcatacatggacatcagtggcctaagattcgacgacacggccgtctattactgtgcgagagatcgctcctatgacgactcctcttgggccttagatgcctggggacagggaacgacggtcgtcgtctccgcg

SEQ ID NO: 103 - DNA, 366 bp, Homo sapiens
  source 1..366: mol_type = other DNA
cgagcgcacctggtacaatcagggactgcgatgaagaaaccgggggcctcagtaagagtctcctgccagacctctggatacacctttaccgcccacatattattttggttccgacaggcccccgggcgaggacttgagtgggtggggtggatcaagccacaatatggggccgtgaattttggtggtggttttcgggacagggtcacattgactcgagacatatatagagagattgcgtacatggacatcagaggccttaaacttgacgacacggccgtctattactgtgcgagagaccgttcctatggcgactcctcttgggccttagatgcctggggacagggaacgacggtcgtcgtctccgcg

SEQ ID NO: 104 - protein, 103 aa, Homo sapiens
YIHVTQSPSSLSVSIGDRVTINCQTSQGVGSDLHWYQHKPGRDPKLLIRHTTSVEDGVPSRVSGSGFHTSFNLTISDLQADDIATYYCQVLQFFGRGSRLHIK

SEQ ID NO: 105 - DNA, 309 bp, Homo sapiens
  source 1..309: mol_type = other DNA
tacatccacgtgacccagtctccgtcctccctgtctgtgtctattggagacagagtcaccatcaattgccagacgagtcagggtgttggcagtgacctacattggtatcaacacaaaccggggagagaccctaaactcttgatccgccataccacttctgtggaagacggtgtcccctcaagagtcagcggctctggatttcacacatcttttaatctgaccatcagcgacctacaggctgacgacattgccacatattactgtcaagttttacaatttttcggccgagggagtcgactccatattaaa

SEQ ID NO: 106 - protein, 103 aa, Homo sapiens
YIHVTQSPSSLSVSIGDRVTINCQTSQGVGSDLHWYQHKPGRAPKLLIHHASSVDDGVPSRFSGSGFHTSFNLTINDLQADDIATYYCQVLQFFGRGSRLHIK

SEQ ID NO: 107 - DNA, 309 bp, Homo sapiens
  source 1..309: mol_type = other DNA
tacatccacgtgacccagtctccgtcctccctgtctgtgtctattggagacagggtcaccatcaattgccagacgagtcagggtgttggcagtgacctacattggtatcaacacaagccggggagagcccctaaactcttgattcatcatgcctcttctgtggacgacggtgtcccgtcaagattcagtggctctggatttcacacatcttttaatctgaccatcaacgacctacaggctgacgacattgccacatattactgtcaggttttacaatttttcggccgagggagtcgactccatattaaa

SEQ ID NO: 108 - protein, 103 aa, Homo sapiens
YIHVTQSPSSLSVSIGDRVTINCQTSQGVGSDLHWYQHKPGRAPKLLIHHASSVEDGVPSRFSGTGFHTSFNLTINDLQADDIGTYYCQVLQSFGRGSRLDTK

SEQ ID NO: 109 - DNA, 309 bp, Homo sapiens
  source 1..309: mol_type = other DNA
tacatccacgtgacccagtctccgtcctccctgtctgtgtctataggggacagagtcaccatcaattgccagacgagtcagggtgttggcagtgacctacattggtatcaacacaaaccggggagagcccctaaactcctgatccaccatgcctcttctgtggaggacggtgtcccgtcaagattcagtggcactggatttcacacatcttttaatttgaccatcaacgacctgcaggctgacgacattggcacttattactgtcaggtgttacaatctttcggccgagggagtcgactggatactaaa

SEQ ID NO: 110 - protein, 103 aa, Homo sapiens
YIHVTQSPSSLSVSIGDRVTINCQTSQGFGRDLHWYQHKPGRAPKLLIHHAPYVDDGVPSRFSGSGFHTSFNLTINDLQADDIATYYCQVLQFFGRGSRLHIK

SEQ ID NO: 111 - DNA, 309 bp, Homo sapiens
  source 1..309: mol_type = other DNA
tacatccacgtgacccagtctccgtcctccctgtctgtgtctattggagacagggtcaccatcaattgccagacgagtcagggttttggcagggacctacattggtatcaacacaagccggggagagcccctaaactcttgattcatcatgccccttatgtggacgacggtgtcccttcaagattcagtggctctggatttcacacatcttttaatctgaccatcaacgacctacaggctgacgacattgccacatattactgtcaggttttacaatttttcggccgagggagtcgactccatattaaa

SEQ ID NO: 112 - protein, 121 aa, Homo sapiens
RAHLVQSGTAMKKPGASVRVSCQTSGYTFTAHILFWFRQAPGRGLEWVGWIKPQYGAVNFGGGFRDRVTLTRDIYREIAYMDIRGLKLDDTAVYYCARDRSYGDSSWALDAWGQGTTVVVS

SEQ ID NO: 113 - DNA, 363 bp, Homo sapiens
  source 1..363: mol_type = other DNA
cgagcgcacctggtacaatcagggactgcgatgaagaaaccgggggcctcagtaagggtctcctgccagacttctggatacacctttaccgcccacatattattttggttccgacaggcccccgggcgagggctggagtgggtgggatggatcaagccacaatacggggccgtgaattttggtggtggttttcgggacagggtcacattgactcgagacatatatagagagattgcatacatggacatcagaggccttaaacttgacgacacggccgtctattactgtgcgagagaccgttcctatggcgactcctcttgggccttagatgcctggggacagggaacgacggtcgtcgtctcc

SEQ ID NO: 114 - protein, 122 aa, Homo sapiens
RAHLVQSGTAMKKPGASVRVSCQTSGYTFTAHILFWFRQAPGRGLEWVGWIKPQYGAVNFGGGFRDRVTLTRDIYREIAYMDIRGLKLDDTAVYYCARDRSYGDSSWALDAWGQGTTVVVSA

SEQ ID NO: 115 - DNA, 366 bp, Homo sapiens
  source 1..366: mol_type = other DNA
cgagcgcacctggtacaatcagggactgcgatgaagaaaccgggggcctcagtaagggtctcctgccagacttctggatacacctttaccgcccacatattattttggttccgacaggcccccgggcgagggctggagtgggtgggatggatcaagccacaatacggggccgtgaattttggtggtggttttcgggacagggtcacattgactcgagacatatatagagagattgcatacatggacatcagaggccttaaacttgacgacacggccgtctattactgtgcgagagaccgttcctatggcgactcctcttgggccttagatgcctggggacagggaacgacggtcgtcgtctccgcg